European Patent Application EP 4 252 782 A1, published October 4, 2023. Title: ANTI-CLDN18.2 ANTIBODY, DRUG CONJUGATE, AND PREPARATION METHOD THEREFOR AND USE THEREOF. Applicant: CSPC MEGALITH BIOPHARMACEUTICAL CO., LTD. Application EP21897116.6. The sequence listing filed with the application follows.

SEQUENCE LISTING (20 sequences)

SEQ ID NO: 1 - protein, 8 aa, Artificial Sequence
  HCDR1
GFTFSSYA

SEQ ID NO: 2 - protein, 8 aa, Artificial Sequence
  HCDR2
LSGSGRST

SEQ ID NO: 3 - protein, 13 aa, Artificial Sequence
  HCDR3
AKSLSYYHYYFDY

SEQ ID NO: 4 - protein, 6 aa, Artificial Sequence
  LCDR1
QDISNY

SEQ ID NO: 5 - protein, 3 aa, Artificial Sequence
  LCDR2
SAS

SEQ ID NO: 6 - protein, 9 aa, Artificial Sequence
  LCDR3
QQVKTYPLT

SEQ ID NO: 7 - protein, 120 aa, Artificial Sequence
  Heavy Chain Variable Region
EVQLSESGGALVQPGESLRLSCAASGFTFSSYAMTWVRQAPGKGLEWVSSLSGSGRSTYYAASIKGRFTISRDNSKNTLYLQMSSLRAEDTAIYYCAKSLSYYHYYFDYWGQGTLVTVSS

SEQ ID NO: 8 - protein, 107 aa, Artificial Sequence
  Light Chain Variable Region
DIQLTQSPSFLSASVGDRVPITCRASQDISNYLAWYQQKPGKAPKLLIYSASTLQSGVPSRFSGSGSGTEFTLTISSLQPEDFASYHCQQVKTYPLTFGGGTKVEIK

SEQ ID NO: 9 - protein, 450 aa, Artificial Sequence
  Heavy Chain
EVQLSESGGALVQPGESLRLSCAASGFTFSSYAMTWVRQAPGKGLEWVSSLSGSGRSTYYAASIKGRFTISRDNSKNTLYLQMSSLRAEDTAIYYCAKSLSYYHYYFDYWGQGTLVTVSSASTKGPSVFPLAPSSKSTSGGTAALGCLVKDYFPEPVTVSWNSGALTSGVHTFPAVLQSSGLYSLSSVVTVPSSSLGTQTYICNVNHKPSNTKVDKKVEPKSCDKTHTCPPCPAPELLGGPSVFLFPPKPKDTLMISRTPEVTCVVVDVSHEDPEVKFNWYVDGVEVHNAKTKPREEQYNSTYRVVSVLTVLHQDWLNGKEYKCKVSNKALPAPIEKTISKAKGQPREPQVYTLPPSRDELTKNQVSLTCLVKGFYPSDIAVEWESNGQPENNYKTTPPVLDSDGSFFLYSKLTVDKSRWQQGNVFSCSVMHEALHNHYTQKSLSLSPGK

SEQ ID NO: 10 - protein, 214 aa, Artificial Sequence
  Light Chain
DIQLTQSPSFLSASVGDRVPITCRASQDISNYLAWYQQKPGKAPKLLIYSASTLQSGVPSRFSGSGSGTEFTLTISSLQPEDFASYHCQQVKTYPLTFGGGTKVEIKRTVAAPSVFIFPPSDEQLKSGTASVVCLLNNFYPREAKVQWKVDNALQSGNSQESVTEQDSKDSTYSLSSTLTLSKADYEKHKVYACEVTHQGLSSPVTKSFNRGEC

SEQ ID NO: 11 - protein, 25 aa, Artificial Sequence
  FR-H1
EVQLSESGGALVQPGESLRLSCAAS

SEQ ID NO: 12 - protein, 17 aa, Artificial Sequence
  FR-H2
MTWVRQAPGKGLEWVSS

SEQ ID NO: 13 - protein, 38 aa, Artificial Sequence
  FR-H3
YYAASIKGRFTISRDNSKNTLYLQMSSLRAEDTAIYYC

SEQ ID NO: 14 - protein, 11 aa, Artificial Sequence
  FR-H4
WGQGTLVTVSS

SEQ ID NO: 15 - protein, 26 aa, Artificial Sequence
  FR-L1
DIQLTQSPSFLSASVGDRVPITCRAS

SEQ ID NO: 16 - protein, 17 aa, Artificial Sequence
  FR-L2
LAWYQQKPGKAPKLLIY

SEQ ID NO: 17 - protein, 36 aa, Artificial Sequence
  FR-L3
TLQSGVPSRFSGSGSGTEFTLTISSLQPEDFASYHC

SEQ ID NO: 18 - protein, 10 aa, Artificial Sequence
  FR-L4
FGGGTKVEIK

SEQ ID NO: 19 - protein, 19 aa, Artificial Sequence
  signal peptide sequence
MGWSCIILFLVATATGVHS

SEQ ID NO: 20 - protein, 331 aa, Artificial Sequence
  amino acid seqeucne of transglutaminase
DSDERVTPPAEPLDRMPDPYRPSYGRAETIVNNYIRKWQQVYSHRDGRKQQMTEEQREWLSYGCVGVTWVNSGQYPTNRLAFAFFDEDKYKNELKNGRPRSGETRAEFEGRVAKDSFDEAKGFQRARDVASVMNKALENAHDEGAYLDNLKKELANGNDALRNEDARSPFYSALRNTPSFKDRNGGNHDPSKMKAVIYSKHFWSGQDRSGSSDKRKYGDPEAFRPDRGTGLVDMSRDRNIPRSPTSPGESFVNFDYGWFGAQTEADADKTVWTHGNHYHAPNGSLGAMHVYESKFRNWSDGYSDFDRGAYVVTFVPKSWNTAPDKVTQGWP